European Patent Application EP 4 238 990 A1, published September 6, 2023. Title: FULLY HUMAN ANTIBODY TARGETING CD5, FULLY HUMAN CHIMERIC ANTIGEN RECEPTOR (CAR) AND APPLICATION THEREOF. Applicant: Nanjing IASO Biotherapeutics Co., Ltd. The sequence listing filed with the application follows.

SEQUENCE LISTING (106 sequences)

SEQ ID NO: 1 - DNA, 63 bp, Artificial sequence
  CD8a signal nucleic acid sequence
atggccctgcctgtgacagctctgctcctccctctggccctgctgctccatgccgccagaccc

SEQ ID NO: 2 - protein, 21 aa, Artificial sequence
  CD8a signal protein sequence
MALPVTALLLPLALLLHAARP

SEQ ID NO: 3 - DNA, 165 bp, Artificial sequence
  CD8a hinge nucleic acid sequence
ttcgtgcccgtgttcctgcccgccaaacctactactacccctgcacctaggcctcccaccccagccccaacaatcgccagccagcctctgtctctgcggcccgaagcctgtagacctgctgccggcggagccgtgcacaccagaggcctggacttcgcctgcgac

SEQ ID NO: 4 - protein, 55 aa, Artificial sequence
  CD8a hinge protein sequence
FVPVFLPAKPTTTPAPRPPTPAPTIASQPLSLRPEACRPAAGGAVHTRGLDFACD

SEQ ID NO: 5 - DNA, 84 bp, Artificial sequence
  CD8a TM nucleic acid sequence
atctacatctgggcccctctggccggcacctgtggcgtgctgctgctgagcctggtgatcaccctgtactgcaaccaccggaac

SEQ ID NO: 6 - protein, 28 aa, Artificial sequence
  CD8a TM protein sequence
IYIWAPLAGTCGVLLLSLVITLYCNHRN

SEQ ID NO: 7 - DNA, 126 bp, Artificial sequence
  4-1BB intracellular domain nucleic acid sequence
aaacggggcagaaagaaactcctgtatatattcaaacaaccatttatgagaccagtacaaactactcaagaggaagatggctgtagctgccgatttccagaagaagaagaaggaggatgtgaactg

SEQ ID NO: 8 - protein, 42 aa, Artificial sequence
  4-1BB intracellular domain protein sequence
KRGRKKLLYIFKQPFMRPVQTTQEEDGCSCRFPEEEEGGCEL

SEQ ID NO: 9 - DNA, 336 bp, Artificial sequence
  CD3ζz intracellular signaling domain nucleic acid sequence
agagtgaagttcagcagatccgccgacgcccctgcctaccagcagggacagaaccagctgtacaacgagctgaacctgggcagacgggaagagtacgacgtgctggacaagcggagaggccgggaccccgagatgggcggaaagcccagacggaagaacccccaggaaggcctgtataacgaactgcagaaagacaagatggccgaggcctacagcgagatcggcatgaagggcgagcggaggcgcggcaagggccacgatggcctgtaccagggcctgagcaccgccaccaaggacacctacgacgccctgcacatgcaggccctgccccccaga

SEQ ID NO: 10 - protein, 112 aa, Artificial sequence
  CD3ζz intracellular signaling domain protein sequence
RVKFSRSADAPAYQQGQNQLYNELNLGRREEYDVLDKRRGRDPEMGGKPRRKNPQEGLYNELQKDKMAEAYSEIGMKGERRRGKGHDGLYQGLSTATKDTYDALHMQALPPR

SEQ ID NO: 11 - DNA, 54 bp, Artificial sequence
  Splicing peptide T2A nucleic acid sequence
gagggaaggggcagcttattaacatgtggcgatgtggaagagaaccccggtccc

SEQ ID NO: 12 - protein, 18 aa, Artificial sequence
  Splicing peptide T2A protein sequence
EGRGSLLTCGDVEENPGP

SEQ ID NO: 13 - DNA, 66 bp, Artificial sequence
  CSF2RA signal nucleic acid sequence
atgctgctgctcgtgacctctttactgttatgtgagctgccccaccccgcttttttactgatccct

SEQ ID NO: 14 - protein, 22 aa, Artificial sequence
  CSF2RA signal protein sequence
MLLLVTSLLLCELPHPAFLLIP

SEQ ID NO: 15 - DNA, 1005 bp, Artificial sequence
  tEGFR nucleic acid sequence
cgtaaggtgtgtaacggaatcggcattggcgagttcaaggactctttaagcatcaacgccacaaacatcaagcacttcaagaattgtacctccatcagcggcgatttacacattctccccgtggcttttcgtggcgattccttcacccacaccccccctctggacccccaagagctggacattttaaaaaccgtgaaggagatcaccggctttctgctgatccaagcttggcccgagaatcgtaccgacctccacgccttcgagaatttagagattattcgtggaaggaccaagcagcacggccagttctctttagccgtcgtgtctttaaacattaccagcctcggtttaaggtctttaaaggagattagcgacggcgacgtgatcatctccggcaacaagaacctctgctacgccaacaccatcaactggaagaagctgttcggaaccagcggccaaaagaccaagatcatcagcaatcgtggagagaactcttgtaaggccactggtcaagtttgccacgccctctgtagccccgaaggatgttggggccccgagcctagggactgtgttagctgcagaaacgtgagcagaggcagagagtgtgtggacaaatgcaatttactggaaggagagcctagggagttcgtggagaacagcgaatgtatccagtgccaccccgagtgtttacctcaagccatgaacatcacttgtaccggaaggggccccgataactgcatccaatgcgcccactacatcgacggaccccactgcgtgaaaacttgtcccgccggagtgatgggagagaataacactttagtgtggaagtacgccgacgctggccacgtctgccatctgtgccaccccaactgtacctacggctgcactggtcccggtttagagggatgtcctaccaacggccccaagatcccctccatcgccaccggaatggtgggcgctctgttattactgctggtggtggctctgggcatcggtttattcatg

SEQ ID NO: 16 - protein, 335 aa, Artificial sequence
  tEGFR protein sequence
RKVCNGIGIGEFKDSLSINATNIKHFKNCTSISGDLHILPVAFRGDSFTHTPPLDPQELDILKTVKEITGFLLIQAWPENRTDLHAFENLEIIRGRTKQHGQFSLAVVSLNITSLGLRSLKEISDGDVIISGNKNLCYANTINWKKLFGTSGQKTKIISNRGENSCKATGQVCHALCSPEGCWGPEPRDCVSCRNVSRGRECVDKCNLLEGEPREFVENSECIQCHPECLPQAMNITCTGRGPDNCIQCAHYIDGPHCVKTCPAGVMGENNTLVWKYADAGHVCHLCHPNCTYGCTGPGLEGCPTNGPKIPSIATGMVGALLLLLVVALGIGLFM

SEQ ID NO: 17 - DNA, 57 bp, Artificial sequence
  VH-VL linker peptide nucleic acid sequence
tctagaggtggtggtggtagcggcggcggcggctctggtggtggtggatccctcgag

SEQ ID NO: 18 - protein, 19 aa, Artificial sequence
  VH-VL linker peptide protein sequence
SRGGGGSGGGGSGGGGSLE

SEQ ID NO: 19 - DNA, 2658 bp, Artificial sequence
  CAR001 nucleic acid sequence
atggccctgcctgtgacagctctgctcctccctctggccctgctgctccatgccgccagaccccagtctgtcgtgacgcagccgccctcagtgtctggggccccagggcagagggtcaccatctcctgcactgggagcagctccaacatcggggcaggttatgatgtacactggtaccagcagcttccaggaacagcccccaaactcctcatctatggtaacatcaatcggccctcgggggtccctgaccgattctctggctccaagtctggcacctcagcctccctggccatcactgggctccaggctgaggatgaggctgattattactgcggaacatgggacaacagcctgagcgcccattatgtcttcggaactgggaccaaggtcaccgtcctaggttctagaggtggtggtggtagcggcggcggcggctctggtggtggtggatccctcgaggaggtgcagctgttggagtctgggggaggcctggtcaagcctggggggtccctgagactctcctgtgcagcctctggattcaccttcaataactataccatgaactgggtccgccaggctccagggaaggggctggagtgggtctcatccattagtagtagtagtagttacatctactacgcagactcagtgaagggccgattcaccatctccagagacaacgccaagaactcactgtttctgcaaatgaacagcctgagaggcgaggacacggccgtgtattactgtgcgcgctacttctctggttctgctggtgattactggggtcaaggtactctggtgaccgtctcctcattcgtgcccgtgttcctgcccgccaaacctactactacccctgcacctaggcctcccaccccagccccaacaatcgccagccagcctctgtctctgcggcccgaagcctgtagacctgctgccggcggagccgtgcacaccagaggcctggacttcgcctgcgacatctacatctgggcccctctggccggcacctgtggcgtgctgctgctgagcctggtgatcaccctgtactgcaaccaccggaacaaacggggcagaaagaaactcctgtatatattcaaacaaccatttatgagaccagtacaaactactcaagaggaagatggctgtagctgccgatttccagaagaagaagaaggaggatgtgaactgagagtgaagttcagcagatccgccgacgcccctgcctaccagcagggacagaaccagctgtacaacgagctgaacctgggcagacgggaagagtacgacgtgctggacaagcggagaggccgggaccccgagatgggcggaaagcccagacggaagaacccccaggaaggcctgtataacgaactgcagaaagacaagatggccgaggcctacagcgagatcggcatgaagggcgagcggaggcgcggcaagggccacgatggcctgtaccagggcctgagcaccgccaccaaggacacctacgacgccctgcacatgcaggccctgccccccagaggatccggagagggaaggggcagcttattaacatgtggcgatgtggaagagaaccccggtcccatgctgctgctcgtgacctctttactgttatgtgagctgccccaccccgcttttttactgatccctcgtaaggtgtgtaacggaatcggcattggcgagttcaaggactctttaagcatcaacgccacaaacatcaagcacttcaagaattgtacctccatcagcggcgatttacacattctccccgtggcttttcgtggcgattccttcacccacaccccccctctggacccccaagagctggacattttaaaaaccgtgaaggagatcaccggctttctgctgatccaagcttggcccgagaatcgtaccgacctccacgccttcgagaatttagagattattcgtggaaggaccaagcagcacggccagttctctttagccgtcgtgtctttaaacattaccagcctcggtttaaggtctttaaaggagattagcgacggcgacgtgatcatctccggcaacaagaacctctgctacgccaacaccatcaactggaagaagctgttcggaaccagcggccaaaagaccaagatcatcagcaatcgtggagagaactcttgtaaggccactggtcaagtttgccacgccctctgtagccccgaaggatgttggggccccgagcctagggactgtgttagctgcagaaacgtgagcagaggcagagagtgtgtggacaaatgcaatttactggaaggagagcctagggagttcgtggagaacagcgaatgtatccagtgccaccccgagtgtttacctcaagccatgaacatcacttgtaccggaaggggccccgataactgcatccaatgcgcccactacatcgacggaccccactgcgtgaaaacttgtcccgccggagtgatgggagagaataacactttagtgtggaagtacgccgacgctggccacgtctgccatctgtgccaccccaactgtacctacggctgcactggtcccggtttagagggatgtcctaccaacggccccaagatcccctccatcgccaccggaatggtgggcgctctgttattactgctggtggtggctctgggcatcggtttattcatg

SEQ ID NO: 20 - DNA, 2652 bp, Artificial sequence
  CAR002 nucleic acid sequence
atggccctgcctgtgacagctctgctcctccctctggccctgctgctccatgccgccagaccccaggtgcagctggtggagtctgggggaggcctggtcaagcctggggggtccctgagactctcctgtgcagcctctggattcaccttcagtagctatagcatgaactgggtccgccaggctccagggaaggggctggagtgggtctcatccattagtagtagtagtagttacatatactacgcagactcagtgaagggccgattcaccatctccagagacaacgccaagaactcactgtatctgcaaatgaacagcctgagagccgaggacacggctgtgtattactgtgcgagaggaaatccgtggtacggagttgactactggggccagggaaccctggtcaccgtctcctcaactagtggtggtggtggtagcggcggcggcggctctggtggtggtggatccgagctccagtctgtgttgacgcagccgccctcagtgtctgcggccccaggacagaaggtcaccatctcctgctctggaagcaactccaatattggcaataattatgtatcctggtaccagcagctcccaggaacagcccccaaacgcctcatttatgacaataataagcgaccctcagggattcctgaccgattctctggctccaagtctggcacgtcagccaccctgggcatcaccggactccagactggggacgaggccgattattactgcggaatatgggatagcagcctggatgcttatgtcttcggaactgggaccaaggtcaccgtcctaggtttcgtgcccgtgttcctgcccgccaaacctactactacccctgcacctaggcctcccaccccagccccaacaatcgccagccagcctctgtctctgcggcccgaagcctgtagacctgctgccggcggagccgtgcacaccagaggcctggacttcgcctgcgacatctacatctgggcccctctggccggcacctgtggcgtgctgctgctgagcctggtgatcaccctgtactgcaaccaccggaacaaacggggcagaaagaaactcctgtatatattcaaacaaccatttatgagaccagtacaaactactcaagaggaagatggctgtagctgccgatttccagaagaagaagaaggaggatgtgaactgagagtgaagttcagcagatccgccgacgcccctgcctaccagcagggacagaaccagctgtacaacgagctgaacctgggcagacgggaagagtacgacgtgctggacaagcggagaggccgggaccccgagatgggcggaaagcccagacggaagaacccccaggaaggcctgtataacgaactgcagaaagacaagatggccgaggcctacagcgagatcggcatgaagggcgagcggaggcgcggcaagggccacgatggcctgtaccagggcctgagcaccgccaccaaggacacctacgacgccctgcacatgcaggccctgccccccagaggatccggagagggaaggggcagcttattaacatgtggcgatgtggaagagaaccccggtcccatgctgctgctcgtgacctctttactgttatgtgagctgccccaccccgcttttttactgatccctcgtaaggtgtgtaacggaatcggcattggcgagttcaaggactctttaagcatcaacgccacaaacatcaagcacttcaagaattgtacctccatcagcggcgatttacacattctccccgtggcttttcgtggcgattccttcacccacaccccccctctggacccccaagagctggacattttaaaaaccgtgaaggagatcaccggctttctgctgatccaagcttggcccgagaatcgtaccgacctccacgccttcgagaatttagagattattcgtggaaggaccaagcagcacggccagttctctttagccgtcgtgtctttaaacattaccagcctcggtttaaggtctttaaaggagattagcgacggcgacgtgatcatctccggcaacaagaacctctgctacgccaacaccatcaactggaagaagctgttcggaaccagcggccaaaagaccaagatcatcagcaatcgtggagagaactcttgtaaggccactggtcaagtttgccacgccctctgtagccccgaaggatgttggggccccgagcctagggactgtgttagctgcagaaacgtgagcagaggcagagagtgtgtggacaaatgcaatttactggaaggagagcctagggagttcgtggagaacagcgaatgtatccagtgccaccccgagtgtttacctcaagccatgaacatcacttgtaccggaaggggccccgataactgcatccaatgcgcccactacatcgacggaccccactgcgtgaaaacttgtcccgccggagtgatgggagagaataacactttagtgtggaagtacgccgacgctggccacgtctgccatctgtgccaccccaactgtacctacggctgcactggtcccggtttagagggatgtcctaccaacggccccaagatcccctccatcgccaccggaatggtgggcgctctgttattactgctggtggtggctctgggcatcggtttattcatg

SEQ ID NO: 21 - DNA, 2664 bp, Artificial sequence
  CAR003 nucleic acid sequence
atggccctgcctgtgacagctctgctcctccctctggccctgctgctccatgccgccagaccccagtctgtgctgacgcagccgccctcagtgtctgcggccccaggacagaaggtcaccatctcctgctctggaagcagctccaacattgggaataattatgtatcctggtaccagcagctcccaggaacagcccccaaactcctcatttatgacaataataagcgaccctcagggattcctgaccgattctctggctccaagtctggcacgtcagccaccctgggcatcaccggactccagactggggacgaggccgattattactgcggaacatgggatagcagcctgagtgccgtggtattcggcggagggaccaagctgaccgtcctaggttctagaggtggtggtggtagcggcggcggcggctctggtggtggtggatccctcgagatggcccaggtgcagctggtggagtctgggggaggcttggtacagcctggggggtccctgagactttcctgtgcagcctctggattcacctttagcagctatgccatgagctgggtccgccagactccagggaaggggctggagtgggtctcaactattactgatagtggtgatatcacatactacacagcctccgtgcagggccggttcaccatctccagagacaattccaagaacacgttgtatctgcaaatgaacagcctgagagccgaggacacggccgtatattactgtgcgcgcatgtcttctcattggtacttctctgcagattactggggtcaaggtactctggtgaccgtctcctcattcgtgcccgtgttcctgcccgccaaacctactactacccctgcacctaggcctcccaccccagccccaacaatcgccagccagcctctgtctctgcggcccgaagcctgtagacctgctgccggcggagccgtgcacaccagaggcctggacttcgcctgcgacatctacatctgggcccctctggccggcacctgtggcgtgctgctgctgagcctggtgatcaccctgtactgcaaccaccggaacaaacggggcagaaagaaactcctgtatatattcaaacaaccatttatgagaccagtacaaactactcaagaggaagatggctgtagctgccgatttccagaagaagaagaaggaggatgtgaactgagagtgaagttcagcagatccgccgacgcccctgcctaccagcagggacagaaccagctgtacaacgagctgaacctgggcagacgggaagagtacgacgtgctggacaagcggagaggccgggaccccgagatgggcggaaagcccagacggaagaacccccaggaaggcctgtataacgaactgcagaaagacaagatggccgaggcctacagcgagatcggcatgaagggcgagcggaggcgcggcaagggccacgatggcctgtaccagggcctgagcaccgccaccaaggacacctacgacgccctgcacatgcaggccctgccccccagaggatccggagagggaaggggcagcttattaacatgtggcgatgtggaagagaaccccggtcccatgctgctgctcgtgacctctttactgttatgtgagctgccccaccccgcttttttactgatccctcgtaaggtgtgtaacggaatcggcattggcgagttcaaggactctttaagcatcaacgccacaaacatcaagcacttcaagaattgtacctccatcagcggcgatttacacattctccccgtggcttttcgtggcgattccttcacccacaccccccctctggacccccaagagctggacattttaaaaaccgtgaaggagatcaccggctttctgctgatccaagcttggcccgagaatcgtaccgacctccacgccttcgagaatttagagattattcgtggaaggaccaagcagcacggccagttctctttagccgtcgtgtctttaaacattaccagcctcggtttaaggtctttaaaggagattagcgacggcgacgtgatcatctccggcaacaagaacctctgctacgccaacaccatcaactggaagaagctgttcggaaccagcggccaaaagaccaagatcatcagcaatcgtggagagaactcttgtaaggccactggtcaagtttgccacgccctctgtagccccgaaggatgttggggccccgagcctagggactgtgttagctgcagaaacgtgagcagaggcagagagtgtgtggacaaatgcaatttactggaaggagagcctagggagttcgtggagaacagcgaatgtatccagtgccaccccgagtgtttacctcaagccatgaacatcacttgtaccggaaggggccccgataactgcatccaatgcgcccactacatcgacggaccccactgcgtgaaaacttgtcccgccggagtgatgggagagaataacactttagtgtggaagtacgccgacgctggccacgtctgccatctgtgccaccccaactgtacctacggctgcactggtcccggtttagagggatgtcctaccaacggccccaagatcccctccatcgccaccggaatggtgggcgctctgttattactgctggtggtggctctgggcatcggtttattcatg

SEQ ID NO: 22 - protein, 886 aa, Artificial sequence
  CAR001 protein sequence
MALPVTALLLPLALLLHAARPQSVVTQPPSVSGAPGQRVTISCTGSSSNIGAGYDVHWYQQLPGTAPKLLIYGNINRPSGVPDRFSGSKSGTSASLAITGLQAEDEADYYCGTWDNSLSAHYVFGTGTKVTVLGSRGGGGSGGGGSGGGGSLEEVQLLESGGGLVKPGGSLRLSCAASGFTFNNYTMNWVRQAPGKGLEWVSSISSSSSYIYYADSVKGRFTISRDNAKNSLFLQMNSLRGEDTAVYYCARYFSGSAGDYWGQGTLVTVSSFVPVFLPAKPTTTPAPRPPTPAPTIASQPLSLRPEACRPAAGGAVHTRGLDFACDIYIWAPLAGTCGVLLLSLVITLYCNHRNKRGRKKLLYIFKQPFMRPVQTTQEEDGCSCRFPEEEEGGCELRVKFSRSADAPAYQQGQNQLYNELNLGRREEYDVLDKRRGRDPEMGGKPRRKNPQEGLYNELQKDKMAEAYSEIGMKGERRRGKGHDGLYQGLSTATKDTYDALHMQALPPRGSGEGRGSLLTCGDVEENPGPMLLLVTSLLLCELPHPAFLLIPRKVCNGIGIGEFKDSLSINATNIKHFKNCTSISGDLHILPVAFRGDSFTHTPPLDPQELDILKTVKEITGFLLIQAWPENRTDLHAFENLEIIRGRTKQHGQFSLAVVSLNITSLGLRSLKEISDGDVIISGNKNLCYANTINWKKLFGTSGQKTKIISNRGENSCKATGQVCHALCSPEGCWGPEPRDCVSCRNVSRGRECVDKCNLLEGEPREFVENSECIQCHPECLPQAMNITCTGRGPDNCIQCAHYIDGPHCVKTCPAGVMGENNTLVWKYADAGHVCHLCHPNCTYGCTGPGLEGCPTNGPKIPSIATGMVGALLLLLVVALGIGLFM

SEQ ID NO: 23 - protein, 884 aa, Artificial sequence
  CAR002 protein sequence
MALPVTALLLPLALLLHAARPQVQLVESGGGLVKPGGSLRLSCAASGFTFSSYSMNWVRQAPGKGLEWVSSISSSSSYIYYADSVKGRFTISRDNAKNSLYLQMNSLRAEDTAVYYCARGNPWYGVDYWGQGTLVTVSSTSGGGGSGGGGSGGGGSELQSVLTQPPSVSAAPGQKVTISCSGSNSNIGNNYVSWYQQLPGTAPKRLIYDNNKRPSGIPDRFSGSKSGTSATLGITGLQTGDEADYYCGIWDSSLDAYVFGTGTKVTVLGFVPVFLPAKPTTTPAPRPPTPAPTIASQPLSLRPEACRPAAGGAVHTRGLDFACDIYIWAPLAGTCGVLLLSLVITLYCNHRNKRGRKKLLYIFKQPFMRPVQTTQEEDGCSCRFPEEEEGGCELRVKFSRSADAPAYQQGQNQLYNELNLGRREEYDVLDKRRGRDPEMGGKPRRKNPQEGLYNELQKDKMAEAYSEIGMKGERRRGKGHDGLYQGLSTATKDTYDALHMQALPPRGSGEGRGSLLTCGDVEENPGPMLLLVTSLLLCELPHPAFLLIPRKVCNGIGIGEFKDSLSINATNIKHFKNCTSISGDLHILPVAFRGDSFTHTPPLDPQELDILKTVKEITGFLLIQAWPENRTDLHAFENLEIIRGRTKQHGQFSLAVVSLNITSLGLRSLKEISDGDVIISGNKNLCYANTINWKKLFGTSGQKTKIISNRGENSCKATGQVCHALCSPEGCWGPEPRDCVSCRNVSRGRECVDKCNLLEGEPREFVENSECIQCHPECLPQAMNITCTGRGPDNCIQCAHYIDGPHCVKTCPAGVMGENNTLVWKYADAGHVCHLCHPNCTYGCTGPGLEGCPTNGPKIPSIATGMVGALLLLLVVALGIGLFM

SEQ ID NO: 24 - protein, 888 aa, Artificial sequence
  CAR003 protein sequence
MALPVTALLLPLALLLHAARPQSVLTQPPSVSAAPGQKVTISCSGSSSNIGNNYVSWYQQLPGTAPKLLIYDNNKRPSGIPDRFSGSKSGTSATLGITGLQTGDEADYYCGTWDSSLSAVVFGGGTKLTVLGSRGGGGSGGGGSGGGGSLEMAQVQLVESGGGLVQPGGSLRLSCAASGFTFSSYAMSWVRQTPGKGLEWVSTITDSGDITYYTASVQGRFTISRDNSKNTLYLQMNSLRAEDTAVYYCARMSSHWYFSADYWGQGTLVTVSSFVPVFLPAKPTTTPAPRPPTPAPTIASQPLSLRPEACRPAAGGAVHTRGLDFACDIYIWAPLAGTCGVLLLSLVITLYCNHRNKRGRKKLLYIFKQPFMRPVQTTQEEDGCSCRFPEEEEGGCELRVKFSRSADAPAYQQGQNQLYNELNLGRREEYDVLDKRRGRDPEMGGKPRRKNPQEGLYNELQKDKMAEAYSEIGMKGERRRGKGHDGLYQGLSTATKDTYDALHMQALPPRGSGEGRGSLLTCGDVEENPGPMLLLVTSLLLCELPHPAFLLIPRKVCNGIGIGEFKDSLSINATNIKHFKNCTSISGDLHILPVAFRGDSFTHTPPLDPQELDILKTVKEITGFLLIQAWPENRTDLHAFENLEIIRGRTKQHGQFSLAVVSLNITSLGLRSLKEISDGDVIISGNKNLCYANTINWKKLFGTSGQKTKIISNRGENSCKATGQVCHALCSPEGCWGPEPRDCVSCRNVSRGRECVDKCNLLEGEPREFVENSECIQCHPECLPQAMNITCTGRGPDNCIQCAHYIDGPHCVKTCPAGVMGENNTLVWKYADAGHVCHLCHPNCTYGCTGPGLEGCPTNGPKIPSIATGMVGALLLLLVVALGIGLFM

SEQ ID NO: 25 - DNA, 750 bp, Artificial sequence
  Scfv10 nucleic acid sequence
cagtctgtcgtgacgcagccgccctcagtgtctggggccccagggcagagggtcaccatctcctgcactgggagcagctccaacatcggggcaggttatgatgtacactggtaccagcagcttccaggaacagcccccaaactcctcatctatggtaacatcaatcggccctcgggggtccctgaccgattctctggctccaagtctggcacctcagcctccctggccatcactgggctccaggctgaggatgaggctgattattactgcggaacatgggacaacagcctgagcgcccattatgtcttcggaactgggaccaaggtcaccgtcctaggttctagaggtggtggtggtagcggcggcggcggctctggtggtggtggatccctcgaggaggtgcagctgttggagtctgggggaggcctggtcaagcctggggggtccctgagactctcctgtgcagcctctggattcaccttcaataactataccatgaactgggtccgccaggctccagggaaggggctggagtgggtctcatccattagtagtagtagtagttacatctactacgcagactcagtgaagggccgattcaccatctccagagacaacgccaagaactcactgtttctgcaaatgaacagcctgagaggcgaggacacggccgtgtattactgtgcgcgctacttctctggttctgctggtgattactggggtcaaggtactctggtgaccgtctcctca

SEQ ID NO: 26 - DNA, 339 bp, Artificial sequence
  10VL (i.e., VL of Scfv10 in CAR001) nucleic acid sequence
cagtctgtcgtgacgcagccgccctcagtgtctggggccccagggcagagggtcaccatctcctgcactgggagcagctccaacatcggggcaggttatgatgtacactggtaccagcagcttccaggaacagcccccaaactcctcatctatggtaacatcaatcggccctcgggggtccctgaccgattctctggctccaagtctggcacctcagcctccctggccatcactgggctccaggctgaggatgaggctgattattactgcggaacatgggacaacagcctgagcgcccattatgtcttcggaactgggaccaaggtcaccgtcctaggt

SEQ ID NO: 27 - DNA, 354 bp, Artificial sequence
  10VH (i.e., VH of Scfv10 in CAR001) nucleic acid sequence
gaggtgcagctgttggagtctgggggaggcctggtcaagcctggggggtccctgagactctcctgtgcagcctctggattcaccttcaataactataccatgaactgggtccgccaggctccagggaaggggctggagtgggtctcatccattagtagtagtagtagttacatctactacgcagactcagtgaagggccgattcaccatctccagagacaacgccaagaactcactgtttctgcaaatgaacagcctgagaggcgaggacacggccgtgtattactgtgcgcgctacttctctggttctgctggtgattactggggtcaaggtactctggtgaccgtctcctca

SEQ ID NO: 28 - protein, 250 aa, Artificial sequence
  Scfv10 protein sequence
QSVVTQPPSVSGAPGQRVTISCTGSSSNIGAGYDVHWYQQLPGTAPKLLIYGNINRPSGVPDRFSGSKSGTSASLAITGLQAEDEADYYCGTWDNSLSAHYVFGTGTKVTVLGSRGGGGSGGGGSGGGGSLEEVQLLESGGGLVKPGGSLRLSCAASGFTFNNYTMNWVRQAPGKGLEWVSSISSSSSYIYYADSVKGRFTISRDNAKNSLFLQMNSLRGEDTAVYYCARYFSGSAGDYWGQGTLVTVSS

SEQ ID NO: 29 - protein, 113 aa, Artificial sequence
  10VL (i.e., VL of Scfv10 in CAR001) protein sequence
QSVVTQPPSVSGAPGQRVTISCTGSSSNIGAGYDVHWYQQLPGTAPKLLIYGNINRPSGVPDRFSGSKSGTSASLAITGLQAEDEADYYCGTWDNSLSAHYVFGTGTKVTVLG

SEQ ID NO: 30 - protein, 118 aa, Artificial sequence
  10VH (i.e., VH of Scfv10 in CAR001) protein sequence
EVQLLESGGGLVKPGGSLRLSCAASGFTFNNYTMNWVRQAPGKGLEWVSSISSSSSYIYYADSVKGRFTISRDNAKNSLFLQMNSLRGEDTAVYYCARYFSGSAGDYWGQGTLVTVSS

SEQ ID NO: 31 - DNA, 744 bp, Artificial sequence
  Scfv32 nucleic acid sequence
caggtgcagctggtggagtctgggggaggcctggtcaagcctggggggtccctgagactctcctgtgcagcctctggattcaccttcagtagctatagcatgaactgggtccgccaggctccagggaaggggctggagtgggtctcatccattagtagtagtagtagttacatatactacgcagactcagtgaagggccgattcaccatctccagagacaacgccaagaactcactgtatctgcaaatgaacagcctgagagccgaggacacggctgtgtattactgtgcgagaggaaatccgtggtacggagttgactactggggccagggaaccctggtcaccgtctcctcaactagtggtggtggtggtagcggcggcggcggctctggtggtggtggatccgagctccagtctgtgttgacgcagccgccctcagtgtctgcggccccaggacagaaggtcaccatctcctgctctggaagcaactccaatattggcaataattatgtatcctggtaccagcagctcccaggaacagcccccaaacgcctcatttatgacaataataagcgaccctcagggattcctgaccgattctctggctccaagtctggcacgtcagccaccctgggcatcaccggactccagactggggacgaggccgattattactgcggaatatgggatagcagcctggatgcttatgtcttcggaactgggaccaaggtcaccgtcctaggt

SEQ ID NO: 32 - DNA, 333 bp, Artificial sequence
  32VL (i.e., VL of Scfv32 in CAR002) nucleic acid sequence
cagtctgtgttgacgcagccgccctcagtgtctgcggccccaggacagaaggtcaccatctcctgctctggaagcaactccaatattggcaataattatgtatcctggtaccagcagctcccaggaacagcccccaaacgcctcatttatgacaataataagcgaccctcagggattcctgaccgattctctggctccaagtctggcacgtcagccaccctgggcatcaccggactccagactggggacgaggccgattattactgcggaatatgggatagcagcctggatgcttatgtcttcggaactgggaccaaggtcaccgtcctaggt

SEQ ID NO: 33 - DNA, 354 bp, Artificial sequence
  32 VH (i.e., VH of Scfv32 in CAR002) nucleic acid sequence
caggtgcagctggtggagtctgggggaggcctggtcaagcctggggggtccctgagactctcctgtgcagcctctggattcaccttcagtagctatagcatgaactgggtccgccaggctccagggaaggggctggagtgggtctcatccattagtagtagtagtagttacatatactacgcagactcagtgaagggccgattcaccatctccagagacaacgccaagaactcactgtatctgcaaatgaacagcctgagagccgaggacacggctgtgtattactgtgcgagaggaaatccgtggtacggagttgactactggggccagggaaccctggtcaccgtctcctca

SEQ ID NO: 34 - protein, 248 aa, Artificial sequence
  Scfv32 protein sequence
QVQLVESGGGLVKPGGSLRLSCAASGFTFSSYSMNWVRQAPGKGLEWVSSISSSSSYIYYADSVKGRFTISRDNAKNSLYLQMNSLRAEDTAVYYCARGNPWYGVDYWGQGTLVTVSSTSGGGGSGGGGSGGGGSELQSVLTQPPSVSAAPGQKVTISCSGSNSNIGNNYVSWYQQLPGTAPKRLIYDNNKRPSGIPDRFSGSKSGTSATLGITGLQTGDEADYYCGIWDSSLDAYVFGTGTKVTVLG

SEQ ID NO: 35 - protein, 111 aa, Artificial sequence
  32 VL (i.e., VL of Scfv32 in CAR002) protein sequence
QSVLTQPPSVSAAPGQKVTISCSGSNSNIGNNYVSWYQQLPGTAPKRLIYDNNKRPSGIPDRFSGSKSGTSATLGITGLQTGDEADYYCGIWDSSLDAYVFGTGTKVTVLG

SEQ ID NO: 36 - protein, 118 aa, Artificial sequence
  32VH (i.e., VH of Scfv32 in CAR002) protein sequence
QVQLVESGGGLVKPGGSLRLSCAASGFTFSSYSMNWVRQAPGKGLEWVSSISSSSSYIYYADSVKGRFTISRDNAKNSLYLQMNSLRAEDTAVYYCARGNPWYGVDYWGQGTLVTVSS

SEQ ID NO: 37 - DNA, 756 bp, Artificial sequence
  Scfv35 nucleic acid sequence
cagtctgtgctgacgcagccgccctcagtgtctgcggccccaggacagaaggtcaccatctcctgctctggaagcagctccaacattgggaataattatgtatcctggtaccagcagctcccaggaacagcccccaaactcctcatttatgacaataataagcgaccctcagggattcctgaccgattctctggctccaagtctggcacgtcagccaccctgggcatcaccggactccagactggggacgaggccgattattactgcggaacatgggatagcagcctgagtgccgtggtattcggcggagggaccaagctgaccgtcctaggttctagaggtggtggtggtagcggcggcggcggctctggtggtggtggatccctcgagatggcccaggtgcagctggtggagtctgggggaggcttggtacagcctggggggtccctgagactttcctgtgcagcctctggattcacctttagcagctatgccatgagctgggtccgccagactccagggaaggggctggagtgggtctcaactattactgatagtggtgatatcacatactacacagcctccgtgcagggccggttcaccatctccagagacaattccaagaacacgttgtatctgcaaatgaacagcctgagagccgaggacacggccgtatattactgtgcgcgcatgtcttctcattggtacttctctgcagattactggggtcaaggtactctggtgaccgtctcctca

SEQ ID NO: 38 - DNA, 333 bp, Artificial sequence
  35VL (i.e., VL of Scfv35 in CAR003) nucleic acid sequence
cagtctgtgctgacgcagccgccctcagtgtctgcggccccaggacagaaggtcaccatctcctgctctggaagcagctccaacattgggaataattatgtatcctggtaccagcagctcccaggaacagcccccaaactcctcatttatgacaataataagcgaccctcagggattcctgaccgattctctggctccaagtctggcacgtcagccaccctgggcatcaccggactccagactggggacgaggccgattattactgcggaacatgggatagcagcctgagtgccgtggtattcggcggagggaccaagctgaccgtcctaggt

SEQ ID NO: 39 - DNA, 366 bp, Artificial sequence
  35VH (i.e., VH of Scfv35 in CAR003) nucleic acid sequence
atggcccaggtgcagctggtggagtctgggggaggcttggtacagcctggggggtccctgagactttcctgtgcagcctctggattcacctttagcagctatgccatgagctgggtccgccagactccagggaaggggctggagtgggtctcaactattactgatagtggtgatatcacatactacacagcctccgtgcagggccggttcaccatctccagagacaattccaagaacacgttgtatctgcaaatgaacagcctgagagccgaggacacggccgtatattactgtgcgcgcatgtcttctcattggtacttctctgcagattactggggtcaaggtactctggtgaccgtctcctca

SEQ ID NO: 40 - protein, 252 aa, Artificial sequence
  Scfv35 protein sequence
QSVLTQPPSVSAAPGQKVTISCSGSSSNIGNNYVSWYQQLPGTAPKLLIYDNNKRPSGIPDRFSGSKSGTSATLGITGLQTGDEADYYCGTWDSSLSAVVFGGGTKLTVLGSRGGGGSGGGGSGGGGSLEMAQVQLVESGGGLVQPGGSLRLSCAASGFTFSSYAMSWVRQTPGKGLEWVSTITDSGDITYYTASVQGRFTISRDNSKNTLYLQMNSLRAEDTAVYYCARMSSHWYFSADYWGQGTLVTVSS

SEQ ID NO: 41 - protein, 111 aa, Artificial sequence
  35 VL (i.e., VL of Scfv35 in CAR003) protein sequence
QSVLTQPPSVSAAPGQKVTISCSGSSSNIGNNYVSWYQQLPGTAPKLLIYDNNKRPSGIPDRFSGSKSGTSATLGITGLQTGDEADYYCGTWDSSLSAVVFGGGTKLTVLG

SEQ ID NO: 42 - protein, 122 aa, Artificial sequence
  35 VH (i.e., VH of Scfv35 in CAR003) protein sequence
MAQVQLVESGGGLVQPGGSLRLSCAASGFTFSSYAMSWVRQTPGKGLEWVSTITDSGDITYYTASVQGRFTISRDNSKNTLYLQMNSLRAEDTAVYYCARMSSHWYFSADYWGQGTLVTVSS

SEQ ID NO: 43 - protein, 8 aa, Artificial sequence
  Amino acid sequence of HCDR1 of Scfv10 (clone 10) antibody in CAR001
GFTFNNYT

SEQ ID NO: 44 - protein, 8 aa, Artificial sequence
  Amino acid sequence of HCDR2 of Scfv10 (clone 10) antibody in CAR001
ISSSSSYI

SEQ ID NO: 45 - protein, 11 aa, Artificial sequence
  Amino acid sequence of HCDR3 of Scfv10 (clone 10) antibody in CAR001
ARYFSGSAGDY

SEQ ID NO: 46 - protein, 9 aa, Artificial sequence
  Amino acid sequence of LCDR1 of Scfv10 (clone 10) antibody in CAR001
SSNIGAGYD

SEQ ID NO: 47 - protein, 3 aa, Artificial Sequence
  Amino acid sequence of LCDR2 of Scfv10 (clone 10) antibody in CAR001
GNI

SEQ ID NO: 48 - protein, 12 aa, Artificial sequence
  Amino acid sequence of LCDR3 of Scfv10 (clone 10) antibody in CAR001
GTWDNSLSAHYV

SEQ ID NO: 49 - protein, 8 aa, Artificial sequence
  Amino acid sequence of HCDR1 of Scfv32 (clone 32) antibody in CAR002
GFTFSSYS

SEQ ID NO: 50 - protein, 8 aa, Artificial sequence
  Amino acid sequence of HCDR2 of Scfv32 (clone 32) antibody in CAR002
ISSSSSYI

SEQ ID NO: 51 - protein, 11 aa, Artificial Sequence
  Amino acid sequence of HCDR3 of Scfv32 (clone 32) antibody in CAR002
ARYFSGSAGDY

SEQ ID NO: 52 - protein, 8 aa, Artificial Sequence
  Amino acid sequence of LCDR1 of Scfv32 (clone 32) antibody in CAR002
NSNIGNNY

SEQ ID NO: 53 - protein, 3 aa, Artificial Sequence
  Amino acid sequence of LCDR2 of Scfv32 (clone 32) antibody in CAR002
DNN

SEQ ID NO: 54 - protein, 11 aa, Artificial sequence
  Amino acid sequence of LCDR3 of Scfv32 (clone 32) antibody in CAR002
GIWDSSLDAYV

SEQ ID NO: 55 - protein, 8 aa, Artificial sequence
  Amino acid sequence of HCDR1 of Scfv35 (clone 35) antibody in CAR003
GFTFSSYA

SEQ ID NO: 56 - protein, 8 aa, Artificial sequence
  Amino acid sequence of HCDR2 of Scfv35 (clone 35) antibody in CAR003
ITDSGDIT

SEQ ID NO: 57 - protein, 13 aa, Artificial sequence
  Amino acid sequence of HCDR3 of Scfv35 (clone 35) antibody in CAR003
ARMSSHWYFSADY

SEQ ID NO: 58 - protein, 8 aa, Artificial sequence
  Amino acid sequence of LCDR1 of Scfv35 (clone 35) antibody in CAR003
SSNIGNNY

SEQ ID NO: 59 - protein, 3 aa, Artificial Sequence
  Amino acid sequence of LCDR2 of Scfv35 (clone 35) antibody in CAR003
DNN

SEQ ID NO: 60 - protein, 11 aa, Artificial sequence
  Amino acid sequence of LCDR3 of Scfv35 (clone 35) antibody in CAR003
GTWDSSLSAVV

SEQ ID NO: 61 - protein, 8 aa, Artificial sequence
  Amino acid sequence of HCDR1 of Scfv6 (clone 6) antibody in CAR004
GGTFSSNA

SEQ ID NO: 62 - protein, 8 aa, Artificial sequence
  Amino acid sequence of HCDR2 of Scfv6 (clone 6) antibody in CAR004
IIPMFGTT

SEQ ID NO: 63 - protein, 17 aa, Artificial sequence
  Amino acid sequence of HCDR3 of Scfv6 (clone 6) antibody in CAR004
ARDGGGRHPYYYYGMDV

SEQ ID NO: 64 - protein, 8 aa, Artificial sequence
  Amino acid sequence of LCDR1 of Scfv6 (clone 6) antibody in CAR004
SGSIARNY

SEQ ID NO: 65 - protein, 3 aa, Artificial Sequence
  Amino acid sequence of LCDR2 of Scfv6 (clone 6) antibody in CAR004
EDN

SEQ ID NO: 66 - protein, 10 aa, Artificial sequence
  Amino acid sequence of LCDR3 of Scfv6 (clone 6) antibody in CAR004
QSYDDNTSWV

SEQ ID NO: 67 - protein, 8 aa, Artificial sequence
  Amino acid sequence of HCDR1 of Scfv7 (clone 7) antibody in CAR005
GYSFTSYW

SEQ ID NO: 68 - protein, 8 aa, Artificial sequence
  Amino acid sequence of HCDR2 of Scfv7 (clone 7) antibody in CAR005
IYPDDSDT

SEQ ID NO: 69 - protein, 13 aa, Artificial sequence
  Amino acid sequence of HCDR3 of Scfv7 (clone 7) antibody in CAR005
ARMSLTSYLATDG

SEQ ID NO: 70 - protein, 8 aa, Artificial sequence
  Amino acid sequence of LCDR1 of Scfv7 (clone 7) antibody in CAR005
SSNIGNND

SEQ ID NO: 71 - protein, 3 aa, Artificial Sequence
  Amino acid sequence of LCDR2 of Scfv7 (clone 7) antibody in CAR005
DND

SEQ ID NO: 72 - protein, 11 aa, Artificial sequence
  Amino acid sequence of LCDR3 of Scfv7 (clone 7) antibody in CAR005
AVWDSSLSAAV

SEQ ID NO: 73 - protein, 8 aa, Artificial sequence
  Amino acid sequence of HCDR1 of Scfv9 (clone 9) antibody in CAR006
TYTFTNYY

SEQ ID NO: 74 - protein, 8 aa, Artificial sequence
  Amino acid sequence of HCDR2 of Scfv9 (clone 9) antibody in CAR006
INPSGDTT

SEQ ID NO: 75 - protein, 13 aa, Artificial sequence
  Amino acid sequence of HCDR3 of Scfv9 (clone 9) antibody in CAR006
ARLSWYWGGSFDD

SEQ ID NO: 76 - protein, 9 aa, Artificial sequence
  Amino acid sequence of LCDR1 of Scfv9 (clone 9) antibody in CAR006
SDDIGNYKR

SEQ ID NO: 77 - protein, 3 aa, Artificial Sequence
  Amino acid sequence of LCDR2 of Scfv9 (clone 9) antibody in CAR006
EVT

SEQ ID NO: 78 - protein, 10 aa, Artificial sequence
  Amino acid sequence of LCDR3 of Scfv9 (clone 9) antibody in CAR006
SSYASGDTYV

SEQ ID NO: 79 - DNA, 771 bp, Artificial sequence
  ScFv6 DNA sequence
aattttatgctgactcagccccactctgtgtcggagtctccggggaagacggtaaccatctcctgcaccggcaatagtggcagcattgccagaaactatgtgcagtggtaccaacagcgcccgggcagtgcccccaccatgctgatctatgaggataatcgaagaccctctggggtccctgatcggttctctggctccatcgacagctcctccaactctgcctccctcaccatctctggactgaagactgaggacgaggctgactattactgtcagtcttatgatgacaacacttcttgggtgttcggcggagggaccaagctgaccgtcctaggttctagaggtggtggtggtagcggcggcggcggctctggtggtggtggatccctcgagatggccgaggtccagctggtacagtctggggctgaggtgaagaagcctgggtcctcggtgaaggtctcctgcaaggcttctggagggaccttcagcagtaatgctatcacctgggtgcgacaggcccctggacaaggccttgagtggatgggagggatcatccctatgtttggtacaacagactacgcacagaagttccagggcagagtcacgatgaccgcggacgaatccacgagcacagcctacatggaactgcgcagcctgagatctgaagacacggccgtgtattactgtgcgagagatggggggggacgacacccctactactactacggtatggacgtctggggccaagggaccacggtcaccgtctcctca

SEQ ID NO: 80 - DNA, 336 bp, Artificial sequence
  6VL (i.e., VL of Scfv6 in CAR004) DNA sequence
aattttatgctgactcagccccactctgtgtcggagtctccggggaagacggtaaccatctcctgcaccggcaatagtggcagcattgccagaaactatgtgcagtggtaccaacagcgcccgggcagtgcccccaccatgctgatctatgaggataatcgaagaccctctggggtccctgatcggttctctggctccatcgacagctcctccaactctgcctccctcaccatctctggactgaagactgaggacgaggctgactattactgtcagtcttatgatgacaacacttcttgggtgttcggcggagggaccaagctgaccgtcctaggt

SEQ ID NO: 81 - DNA, 378 bp, Artificial sequence
  6VH (i.e., VH of Scfv6 in CAR004) DNA sequence
atggccgaggtccagctggtacagtctggggctgaggtgaagaagcctgggtcctcggtgaaggtctcctgcaaggcttctggagggaccttcagcagtaatgctatcacctgggtgcgacaggcccctggacaaggccttgagtggatgggagggatcatccctatgtttggtacaacagactacgcacagaagttccagggcagagtcacgatgaccgcggacgaatccacgagcacagcctacatggaactgcgcagcctgagatctgaagacacggccgtgtattactgtgcgagagatggggggggacgacacccctactactactacggtatggacgtctggggccaagggaccacggtcaccgtctcctca

SEQ ID NO: 82 - DNA, 756 bp, Artificial sequence
  ScFv7 DNA sequence
cagtctgtcgtgacgcagccgccctcagtgtctgcggccccaggacagaaggccaccatctcctgctctggaagcagctccaacattgggaataatgatgtatcctggtaccagcagcttccaggaacagcccccaaactcctcattcaggacaatgataagcgaccctcaggtattcctgaccgattctctggctccaagtctggcacgtcagccaccctgggcatcaccggactccagactggggacgaggccgattattactgcgcagtatgggatagcagcctgagtgctgccgtcttcggacctgggaccaaggtcaccgtcctaggttctagaggtggtggtggtagcggcggcggcggctctggtggtggtggatccctcgagatggccgaagtgcagctggtgcagtctggagcagaggtgaaaaagcccggggagtctctgaagatctcctgtaagggttctggatacagctttaccagctactggatcggctgggtgcgccagatgcccgggaaaggcctggagtggatgggaatcatctatcctgatgactctgataccacgtacagcccgtccttccaaggccaggtcaccatgtcagtcgacaagtccatcagcaccgcctacctgcagtggaacagcctgcaggcctcggacaccgccatgtattactgtgcgcgcatgtctctgacctcttacctggcaaccgatggttggggtcaaggtactctggtgaccgtctcctca

SEQ ID NO: 83 - DNA, 333 bp, Artificial sequence
  7VL (i.e., VL of Scfv7 in CAR005) DNA sequence
cagtctgtcgtgacgcagccgccctcagtgtctgcggccccaggacagaaggccaccatctcctgctctggaagcagctccaacattgggaataatgatgtatcctggtaccagcagcttccaggaacagcccccaaactcctcattcaggacaatgataagcgaccctcaggtattcctgaccgattctctggctccaagtctggcacgtcagccaccctgggcatcaccggactccagactggggacgaggccgattattactgcgcagtatgggatagcagcctgagtgctgccgtcttcggacctgggaccaaggtcaccgtcctaggt

SEQ ID NO: 84 - DNA, 366 bp, Artificial sequence
  7VH (i.e., VH of Scfv7 in CAR005) DNA sequence
atggccgaagtgcagctggtgcagtctggagcagaggtgaaaaagcccggggagtctctgaagatctcctgtaagggttctggatacagctttaccagctactggatcggctgggtgcgccagatgcccgggaaaggcctggagtggatgggaatcatctatcctgatgactctgataccacgtacagcccgtccttccaaggccaggtcaccatgtcagtcgacaagtccatcagcaccgcctacctgcagtggaacagcctgcaggcctcggacaccgccatgtattactgtgcgcgcatgtctctgacctcttacctggcaaccgatggttggggtcaaggtactctggtgaccgtctcctca

SEQ ID NO: 85 - DNA, 750 bp, Artificial sequence
  ScFv9 DNA sequence
cagcctgtgctgactcagcctccctccgtgtccgggtctcctggacagtcagtcaccatctcctgcactggaaccagcgatgacattggaaattataagcgtgtctcctggtaccagcagccccctggcacagcccccaaactcatgatttatgaggtcactaatcggcccccaggggtccctaatcgcttctctgggtccaagtctggcaacacggcctccctgaccatctctgggctccaggctgaggacgaggctgattattactgcagctcatatgcaagcggcgacacttatgtcttcggaactgggaccaaggtcaccgtcctaggttctagaggtggtggtggtagcggcggcggcggctctggtggtggtggatccctcgagcaggtgcagctggtgcagtctggggctgaggtggagaagcctggggcctcagtgaagatttcctgcaaggcatctacatacaccttcaccaactactatatacactgggtacgacaggcccctggacaagggcttgagtggatgggaatgatcaaccctagtggtgataccacaagctacgcacagaagttccagggcagagtcaccatgaccagggacacgtccacgagcactgtctacatggagttgagcagcctgagatctgaggacacggccgtgtattactgtgcgcgcctgtcttggtactggggtggttctttcgatgactggggtcaaggtactctggtgaccgtctcctca

SEQ ID NO: 86 - DNA, 333 bp, Artificial sequence
  9VL (i.e., VL of Scfv9 in CAR006) DNA sequence
cagcctgtgctgactcagcctccctccgtgtccgggtctcctggacagtcagtcaccatctcctgcactggaaccagcgatgacattggaaattataagcgtgtctcctggtaccagcagccccctggcacagcccccaaactcatgatttatgaggtcactaatcggcccccaggggtccctaatcgcttctctgggtccaagtctggcaacacggcctccctgaccatctctgggctccaggctgaggacgaggctgattattactgcagctcatatgcaagcggcgacacttatgtcttcggaactgggaccaaggtcaccgtcctaggt

SEQ ID NO: 87 - DNA, 360 bp, Artificial sequence
  9VH (i.e., VH of Scfv9 in CAR006) DNA sequence
caggtgcagctggtgcagtctggggctgaggtggagaagcctggggcctcagtgaagatttcctgcaaggcatctacatacaccttcaccaactactatatacactgggtacgacaggcccctggacaagggcttgagtggatgggaatgatcaaccctagtggtgataccacaagctacgcacagaagttccagggcagagtcaccatgaccagggacacgtccacgagcactgtctacatggagttgagcagcctgagatctgaggacacggccgtgtattactgtgcgcgcctgtcttggtactggggtggttctttcgatgactggggtcaaggtactctggtgaccgtctcctca

SEQ ID NO: 88 - protein, 257 aa, Artificial sequence
  ScFv6 amino acid sequence
NFMLTQPHSVSESPGKTVTISCTGNSGSIARNYVQWYQQRPGSAPTMLIYEDNRRPSGVPDRFSGSIDSSSNSASLTISGLKTEDEADYYCQSYDDNTSWVFGGGTKLTVLGSRGGGGSGGGGSGGGGSLEMAEVQLVQSGAEVKKPGSSVKVSCKASGGTFSSNAITWVRQAPGQGLEWMGGIIPMFGTTDYAQKFQGRVTMTADESTSTAYMELRSLRSEDTAVYYCARDGGGRHPYYYYGMDVWGQGTTVTVSS

SEQ ID NO: 89 - protein, 112 aa, Artificial sequence
  6VL (i.e., VL of Scfv6 in CAR004) amino acid sequence
NFMLTQPHSVSESPGKTVTISCTGNSGSIARNYVQWYQQRPGSAPTMLIYEDNRRPSGVPDRFSGSIDSSSNSASLTISGLKTEDEADYYCQSYDDNTSWVFGGGTKLTVLG

SEQ ID NO: 90 - protein, 126 aa, Artificial sequence
  6VH (i.e., VH of Scfv6 in CAR004) amino acid sequence
MAEVQLVQSGAEVKKPGSSVKVSCKASGGTFSSNAITWVRQAPGQGLEWMGGIIPMFGTTDYAQKFQGRVTMTADESTSTAYMELRSLRSEDTAVYYCARDGGGRHPYYYYGMDVWGQGTTVTVSS

SEQ ID NO: 91 - protein, 252 aa, Artificial sequence
  ScFv 7 amino acid sequence
QSVVTQPPSVSAAPGQKATISCSGSSSNIGNNDVSWYQQLPGTAPKLLIQDNDKRPSGIPDRFSGSKSGTSATLGITGLQTGDEADYYCAVWDSSLSAAVFGPGTKVTVLGSRGGGGSGGGGSGGGGSLEMAEVQLVQSGAEVKKPGESLKISCKGSGYSFTSYWIGWVRQMPGKGLEWMGIIYPDDSDTTYSPSFQGQVTMSVDKSISTAYLQWNSLQASDTAMYYCARMSLTSYLATDGWGQGTLVTVSS

SEQ ID NO: 92 - protein, 111 aa, Artificial sequence
  7VL (i.e., VL of Scfv7 in CAR005) amino acid sequence
QSVVTQPPSVSAAPGQKATISCSGSSSNIGNNDVSWYQQLPGTAPKLLIQDNDKRPSGIPDRFSGSKSGTSATLGITGLQTGDEADYYCAVWDSSLSAAVFGPGTKVTVLG

SEQ ID NO: 93 - protein, 122 aa, Artificial sequence
  7VH (i.e., VH of Scfv7 in CAR005) amino acid sequence
MAEVQLVQSGAEVKKPGESLKISCKGSGYSFTSYWIGWVRQMPGKGLEWMGIIYPDDSDTTYSPSFQGQVTMSVDKSISTAYLQWNSLQASDTAMYYCARMSLTSYLATDGWGQGTLVTVSS

SEQ ID NO: 94 - protein, 250 aa, Artificial sequence
  ScFv9 amino acid sequence
QPVLTQPPSVSGSPGQSVTISCTGTSDDIGNYKRVSWYQQPPGTAPKLMIYEVTNRPPGVPNRFSGSKSGNTASLTISGLQAEDEADYYCSSYASGDTYVFGTGTKVTVLGSRGGGGSGGGGSGGGGSLEQVQLVQSGAEVEKPGASVKISCKASTYTFTNYYIHWVRQAPGQGLEWMGMINPSGDTTSYAQKFQGRVTMTRDTSTSTVYMELSSLRSEDTAVYYCARLSWYWGGSFDDWGQGTLVTVSS

SEQ ID NO: 95 - protein, 111 aa, Artificial sequence
  9VL (i.e., VL of Scfv9 in CAR006) amino acid sequence
QPVLTQPPSVSGSPGQSVTISCTGTSDDIGNYKRVSWYQQPPGTAPKLMIYEVTNRPPGVPNRFSGSKSGNTASLTISGLQAEDEADYYCSSYASGDTYVFGTGTKVTVLG

SEQ ID NO: 96 - protein, 120 aa, Artificial sequence
  9VH (i.e., VH of Scfv9 in CAR006) amino acid sequence
QVQLVQSGAEVEKPGASVKISCKASTYTFTNYYIHWVRQAPGQGLEWMGMINPSGDTTSYAQKFQGRVTMTRDTSTSTVYMELSSLRSEDTAVYYCARLSWYWGGSFDDWGQGTLVTVSS

SEQ ID NO: 97 - DNA, 2679 bp, Artificial sequence
  CAR004 nucleic acid sequence
atggccctgcctgtgacagctctgctcctccctctggccctgctgctccatgccgccagacccaattttatgctgactcagccccactctgtgtcggagtctccggggaagacggtaaccatctcctgcaccggcaatagtggcagcattgccagaaactatgtgcagtggtaccaacagcgcccgggcagtgcccccaccatgctgatctatgaggataatcgaagaccctctggggtccctgatcggttctctggctccatcgacagctcctccaactctgcctccctcaccatctctggactgaagactgaggacgaggctgactattactgtcagtcttatgatgacaacacttcttgggtgttcggcggagggaccaagctgaccgtcctaggttctagaggtggtggtggtagcggcggcggcggctctggtggtggtggatccctcgagatggccgaggtccagctggtacagtctggggctgaggtgaagaagcctgggtcctcggtgaaggtctcctgcaaggcttctggagggaccttcagcagtaatgctatcacctgggtgcgacaggcccctggacaaggccttgagtggatgggagggatcatccctatgtttggtacaacagactacgcacagaagttccagggcagagtcacgatgaccgcggacgaatccacgagcacagcctacatggaactgcgcagcctgagatctgaagacacggccgtgtattactgtgcgagagatggggggggacgacacccctactactactacggtatggacgtctggggccaagggaccacggtcaccgtctcctcattcgtgcccgtgttcctgcccgccaaacctactactacccctgcacctaggcctcccaccccagccccaacaatcgccagccagcctctgtctctgcggcccgaagcctgtagacctgctgccggcggagccgtgcacaccagaggcctggacttcgcctgcgacatctacatctgggcccctctggccggcacctgtggcgtgctgctgctgagcctggtgatcaccctgtactgcaaccaccggaacaaacggggcagaaagaaactcctgtatatattcaaacaaccatttatgagaccagtacaaactactcaagaggaagatggctgtagctgccgatttccagaagaagaagaaggaggatgtgaactgagagtgaagttcagcagatccgccgacgcccctgcctaccagcagggacagaaccagctgtacaacgagctgaacctgggcagacgggaagagtacgacgtgctggacaagcggagaggccgggaccccgagatgggcggaaagcccagacggaagaacccccaggaaggcctgtataacgaactgcagaaagacaagatggccgaggcctacagcgagatcggcatgaagggcgagcggaggcgcggcaagggccacgatggcctgtaccagggcctgagcaccgccaccaaggacacctacgacgccctgcacatgcaggccctgccccccagaggatccggagagggaaggggcagcttattaacatgtggcgatgtggaagagaaccccggtcccatgctgctgctcgtgacctctttactgttatgtgagctgccccaccccgcttttttactgatccctcgtaaggtgtgtaacggaatcggcattggcgagttcaaggactctttaagcatcaacgccacaaacatcaagcacttcaagaattgtacctccatcagcggcgatttacacattctccccgtggcttttcgtggcgattccttcacccacaccccccctctggacccccaagagctggacattttaaaaaccgtgaaggagatcaccggctttctgctgatccaagcttggcccgagaatcgtaccgacctccacgccttcgagaatttagagattattcgtggaaggaccaagcagcacggccagttctctttagccgtcgtgtctttaaacattaccagcctcggtttaaggtctttaaaggagattagcgacggcgacgtgatcatctccggcaacaagaacctctgctacgccaacaccatcaactggaagaagctgttcggaaccagcggccaaaagaccaagatcatcagcaatcgtggagagaactcttgtaaggccactggtcaagtttgccacgccctctgtagccccgaaggatgttggggccccgagcctagggactgtgttagctgcagaaacgtgagcagaggcagagagtgtgtggacaaatgcaatttactggaaggagagcctagggagttcgtggagaacagcgaatgtatccagtgccaccccgagtgtttacctcaagccatgaacatcacttgtaccggaaggggccccgataactgcatccaatgcgcccactacatcgacggaccccactgcgtgaaaacttgtcccgccggagtgatgggagagaataacactttagtgtggaagtacgccgacgctggccacgtctgccatctgtgccaccccaactgtacctacggctgcactggtcccggtttagagggatgtcctaccaacggccccaagatcccctccatcgccaccggaatggtgggcgctctgttattactgctggtggtggctctgggcatcggtttattcatg

SEQ ID NO: 98 - protein, 893 aa, Artificial sequence
  CAR004 amino acid sequence
MALPVTALLLPLALLLHAARPNFMLTQPHSVSESPGKTVTISCTGNSGSIARNYVQWYQQRPGSAPTMLIYEDNRRPSGVPDRFSGSIDSSSNSASLTISGLKTEDEADYYCQSYDDNTSWVFGGGTKLTVLGSRGGGGSGGGGSGGGGSLEMAEVQLVQSGAEVKKPGSSVKVSCKASGGTFSSNAITWVRQAPGQGLEWMGGIIPMFGTTDYAQKFQGRVTMTADESTSTAYMELRSLRSEDTAVYYCARDGGGRHPYYYYGMDVWGQGTTVTVSSFVPVFLPAKPTTTPAPRPPTPAPTIASQPLSLRPEACRPAAGGAVHTRGLDFACDIYIWAPLAGTCGVLLLSLVITLYCNHRNKRGRKKLLYIFKQPFMRPVQTTQEEDGCSCRFPEEEEGGCELRVKFSRSADAPAYQQGQNQLYNELNLGRREEYDVLDKRRGRDPEMGGKPRRKNPQEGLYNELQKDKMAEAYSEIGMKGERRRGKGHDGLYQGLSTATKDTYDALHMQALPPRGSGEGRGSLLTCGDVEENPGPMLLLVTSLLLCELPHPAFLLIPRKVCNGIGIGEFKDSLSINATNIKHFKNCTSISGDLHILPVAFRGDSFTHTPPLDPQELDILKTVKEITGFLLIQAWPENRTDLHAFENLEIIRGRTKQHGQFSLAVVSLNITSLGLRSLKEISDGDVIISGNKNLCYANTINWKKLFGTSGQKTKIISNRGENSCKATGQVCHALCSPEGCWGPEPRDCVSCRNVSRGRECVDKCNLLEGEPREFVENSECIQCHPECLPQAMNITCTGRGPDNCIQCAHYIDGPHCVKTCPAGVMGENNTLVWKYADAGHVCHLCHPNCTYGCTGPGLEGCPTNGPKIPSIATGMVGALLLLLVVALGIGLFM

SEQ ID NO: 99 - DNA, 2664 bp, Artificial sequence
  CAR005 nucleic acid sequence
atggccctgcctgtgacagctctgctcctccctctggccctgctgctccatgccgccagaccccagtctgtcgtgacgcagccgccctcagtgtctgcggccccaggacagaaggccaccatctcctgctctggaagcagctccaacattgggaataatgatgtatcctggtaccagcagcttccaggaacagcccccaaactcctcattcaggacaatgataagcgaccctcaggtattcctgaccgattctctggctccaagtctggcacgtcagccaccctgggcatcaccggactccagactggggacgaggccgattattactgcgcagtatgggatagcagcctgagtgctgccgtcttcggacctgggaccaaggtcaccgtcctaggttctagaggtggtggtggtagcggcggcggcggctctggtggtggtggatccctcgagatggccgaagtgcagctggtgcagtctggagcagaggtgaaaaagcccggggagtctctgaagatctcctgtaagggttctggatacagctttaccagctactggatcggctgggtgcgccagatgcccgggaaaggcctggagtggatgggaatcatctatcctgatgactctgataccacgtacagcccgtccttccaaggccaggtcaccatgtcagtcgacaagtccatcagcaccgcctacctgcagtggaacagcctgcaggcctcggacaccgccatgtattactgtgcgcgcatgtctctgacctcttacctggcaaccgatggttggggtcaaggtactctggtgaccgtctcctcattcgtgcccgtgttcctgcccgccaaacctactactacccctgcacctaggcctcccaccccagccccaacaatcgccagccagcctctgtctctgcggcccgaagcctgtagacctgctgccggcggagccgtgcacaccagaggcctggacttcgcctgcgacatctacatctgggcccctctggccggcacctgtggcgtgctgctgctgagcctggtgatcaccctgtactgcaaccaccggaacaaacggggcagaaagaaactcctgtatatattcaaacaaccatttatgagaccagtacaaactactcaagaggaagatggctgtagctgccgatttccagaagaagaagaaggaggatgtgaactgagagtgaagttcagcagatccgccgacgcccctgcctaccagcagggacagaaccagctgtacaacgagctgaacctgggcagacgggaagagtacgacgtgctggacaagcggagaggccgggaccccgagatgggcggaaagcccagacggaagaacccccaggaaggcctgtataacgaactgcagaaagacaagatggccgaggcctacagcgagatcggcatgaagggcgagcggaggcgcggcaagggccacgatggcctgtaccagggcctgagcaccgccaccaaggacacctacgacgccctgcacatgcaggccctgccccccagaggatccggagagggaaggggcagcttattaacatgtggcgatgtggaagagaaccccggtcccatgctgctgctcgtgacctctttactgttatgtgagctgccccaccccgcttttttactgatccctcgtaaggtgtgtaacggaatcggcattggcgagttcaaggactctttaagcatcaacgccacaaacatcaagcacttcaagaattgtacctccatcagcggcgatttacacattctccccgtggcttttcgtggcgattccttcacccacaccccccctctggacccccaagagctggacattttaaaaaccgtgaaggagatcaccggctttctgctgatccaagcttggcccgagaatcgtaccgacctccacgccttcgagaatttagagattattcgtggaaggaccaagcagcacggccagttctctttagccgtcgtgtctttaaacattaccagcctcggtttaaggtctttaaaggagattagcgacggcgacgtgatcatctccggcaacaagaacctctgctacgccaacaccatcaactggaagaagctgttcggaaccagcggccaaaagaccaagatcatcagcaatcgtggagagaactcttgtaaggccactggtcaagtttgccacgccctctgtagccccgaaggatgttggggccccgagcctagggactgtgttagctgcagaaacgtgagcagaggcagagagtgtgtggacaaatgcaatttactggaaggagagcctagggagttcgtggagaacagcgaatgtatccagtgccaccccgagtgtttacctcaagccatgaacatcacttgtaccggaaggggccccgataactgcatccaatgcgcccactacatcgacggaccccactgcgtgaaaacttgtcccgccggagtgatgggagagaataacactttagtgtggaagtacgccgacgctggccacgtctgccatctgtgccaccccaactgtacctacggctgcactggtcccggtttagagggatgtcctaccaacggccccaagatcccctccatcgccaccggaatggtgggcgctctgttattactgctggtggtggctctgggcatcggtttattcatg

SEQ ID NO: 100 - protein, 888 aa, Artificial sequence
  CAR005 amino acid sequence
MALPVTALLLPLALLLHAARPQSVVTQPPSVSAAPGQKATISCSGSSSNIGNNDVSWYQQLPGTAPKLLIQDNDKRPSGIPDRFSGSKSGTSATLGITGLQTGDEADYYCAVWDSSLSAAVFGPGTKVTVLGSRGGGGSGGGGSGGGGSLEMAEVQLVQSGAEVKKPGESLKISCKGSGYSFTSYWIGWVRQMPGKGLEWMGIIYPDDSDTTYSPSFQGQVTMSVDKSISTAYLQWNSLQASDTAMYYCARMSLTSYLATDGWGQGTLVTVSSFVPVFLPAKPTTTPAPRPPTPAPTIASQPLSLRPEACRPAAGGAVHTRGLDFACDIYIWAPLAGTCGVLLLSLVITLYCNHRNKRGRKKLLYIFKQPFMRPVQTTQEEDGCSCRFPEEEEGGCELRVKFSRSADAPAYQQGQNQLYNELNLGRREEYDVLDKRRGRDPEMGGKPRRKNPQEGLYNELQKDKMAEAYSEIGMKGERRRGKGHDGLYQGLSTATKDTYDALHMQALPPRGSGEGRGSLLTCGDVEENPGPMLLLVTSLLLCELPHPAFLLIPRKVCNGIGIGEFKDSLSINATNIKHFKNCTSISGDLHILPVAFRGDSFTHTPPLDPQELDILKTVKEITGFLLIQAWPENRTDLHAFENLEIIRGRTKQHGQFSLAVVSLNITSLGLRSLKEISDGDVIISGNKNLCYANTINWKKLFGTSGQKTKIISNRGENSCKATGQVCHALCSPEGCWGPEPRDCVSCRNVSRGRECVDKCNLLEGEPREFVENSECIQCHPECLPQAMNITCTGRGPDNCIQCAHYIDGPHCVKTCPAGVMGENNTLVWKYADAGHVCHLCHPNCTYGCTGPGLEGCPTNGPKIPSIATGMVGALLLLLVVALGIGLFM

SEQ ID NO: 101 - DNA, 2658 bp, Artificial sequence
  CAR006 nucleic acid sequence
atggccctgcctgtgacagctctgctcctccctctggccctgctgctccatgccgccagaccccagcctgtgctgactcagcctccctccgtgtccgggtctcctggacagtcagtcaccatctcctgcactggaaccagcgatgacattggaaattataagcgtgtctcctggtaccagcagccccctggcacagcccccaaactcatgatttatgaggtcactaatcggcccccaggggtccctaatcgcttctctgggtccaagtctggcaacacggcctccctgaccatctctgggctccaggctgaggacgaggctgattattactgcagctcatatgcaagcggcgacacttatgtcttcggaactgggaccaaggtcaccgtcctaggttctagaggtggtggtggtagcggcggcggcggctctggtggtggtggatccctcgagcaggtgcagctggtgcagtctggggctgaggtggagaagcctggggcctcagtgaagatttcctgcaaggcatctacatacaccttcaccaactactatatacactgggtacgacaggcccctggacaagggcttgagtggatgggaatgatcaaccctagtggtgataccacaagctacgcacagaagttccagggcagagtcaccatgaccagggacacgtccacgagcactgtctacatggagttgagcagcctgagatctgaggacacggccgtgtattactgtgcgcgcctgtcttggtactggggtggttctttcgatgactggggtcaaggtactctggtgaccgtctcctcattcgtgcccgtgttcctgcccgccaaacctactactacccctgcacctaggcctcccaccccagccccaacaatcgccagccagcctctgtctctgcggcccgaagcctgtagacctgctgccggcggagccgtgcacaccagaggcctggacttcgcctgcgacatctacatctgggcccctctggccggcacctgtggcgtgctgctgctgagcctggtgatcaccctgtactgcaaccaccggaacaaacggggcagaaagaaactcctgtatatattcaaacaaccatttatgagaccagtacaaactactcaagaggaagatggctgtagctgccgatttccagaagaagaagaaggaggatgtgaactgagagtgaagttcagcagatccgccgacgcccctgcctaccagcagggacagaaccagctgtacaacgagctgaacctgggcagacgggaagagtacgacgtgctggacaagcggagaggccgggaccccgagatgggcggaaagcccagacggaagaacccccaggaaggcctgtataacgaactgcagaaagacaagatggccgaggcctacagcgagatcggcatgaagggcgagcggaggcgcggcaagggccacgatggcctgtaccagggcctgagcaccgccaccaaggacacctacgacgccctgcacatgcaggccctgccccccagaggatccggagagggaaggggcagcttattaacatgtggcgatgtggaagagaaccccggtcccatgctgctgctcgtgacctctttactgttatgtgagctgccccaccccgcttttttactgatccctcgtaaggtgtgtaacggaatcggcattggcgagttcaaggactctttaagcatcaacgccacaaacatcaagcacttcaagaattgtacctccatcagcggcgatttacacattctccccgtggcttttcgtggcgattccttcacccacaccccccctctggacccccaagagctggacattttaaaaaccgtgaaggagatcaccggctttctgctgatccaagcttggcccgagaatcgtaccgacctccacgccttcgagaatttagagattattcgtggaaggaccaagcagcacggccagttctctttagccgtcgtgtctttaaacattaccagcctcggtttaaggtctttaaaggagattagcgacggcgacgtgatcatctccggcaacaagaacctctgctacgccaacaccatcaactggaagaagctgttcggaaccagcggccaaaagaccaagatcatcagcaatcgtggagagaactcttgtaaggccactggtcaagtttgccacgccctctgtagccccgaaggatgttggggccccgagcctagggactgtgttagctgcagaaacgtgagcagaggcagagagtgtgtggacaaatgcaatttactggaaggagagcctagggagttcgtggagaacagcgaatgtatccagtgccaccccgagtgtttacctcaagccatgaacatcacttgtaccggaaggggccccgataactgcatccaatgcgcccactacatcgacggaccccactgcgtgaaaacttgtcccgccggagtgatgggagagaataacactttagtgtggaagtacgccgacgctggccacgtctgccatctgtgccaccccaactgtacctacggctgcactggtcccggtttagagggatgtcctaccaacggccccaagatcccctccatcgccaccggaatggtgggcgctctgttattactgctggtggtggctctgggcatcggtttattcatg

SEQ ID NO: 102 - protein, 886 aa, Artificial Sequence
  CAR006 amino acid sequence
MALPVTALLLPLALLLHAARPQPVLTQPPSVSGSPGQSVTISCTGTSDDIGNYKRVSWYQQPPGTAPKLMIYEVTNRPPGVPNRFSGSKSGNTASLTISGLQAEDEADYYCSSYASGDTYVFGTGTKVTVLGSRGGGGSGGGGSGGGGSLEQVQLVQSGAEVEKPGASVKISCKASTYTFTNYYIHWVRQAPGQGLEWMGMINPSGDTTSYAQKFQGRVTMTRDTSTSTVYMELSSLRSEDTAVYYCARLSWYWGGSFDDWGQGTLVTVSSFVPVFLPAKPTTTPAPRPPTPAPTIASQPLSLRPEACRPAAGGAVHTRGLDFACDIYIWAPLAGTCGVLLLSLVITLYCNHRNKRGRKKLLYIFKQPFMRPVQTTQEEDGCSCRFPEEEEGGCELRVKFSRSADAPAYQQGQNQLYNELNLGRREEYDVLDKRRGRDPEMGGKPRRKNPQEGLYNELQKDKMAEAYSEIGMKGERRRGKGHDGLYQGLSTATKDTYDALHMQALPPRGSGEGRGSLLTCGDVEENPGPMLLLVTSLLLCELPHPAFLLIPRKVCNGIGIGEFKDSLSINATNIKHFKNCTSISGDLHILPVAFRGDSFTHTPPLDPQELDILKTVKEITGFLLIQAWPENRTDLHAFENLEIIRGRTKQHGQFSLAVVSLNITSLGLRSLKEISDGDVIISGNKNLCYANTINWKKLFGTSGQKTKIISNRGENSCKATGQVCHALCSPEGCWGPEPRDCVSCRNVSRGRECVDKCNLLEGEPREFVENSECIQCHPECLPQAMNITCTGRGPDNCIQCAHYIDGPHCVKTCPAGVMGENNTLVWKYADAGHVCHLCHPNCTYGCTGPGLEGCPTNGPKIPSIATGMVGALLLLLVVALGIGLFM

SEQ ID NO: 103 - DNA, 20 bp, Artificial
  sgRNA
aagcgtcaaaagtctgccag

SEQ ID NO: 104 - DNA, 20 bp, Artificial
  sgRNA
ccgttccaactcgaagtgcc

SEQ ID NO: 105 - DNA, 20 bp, Artificial
  sgRNA
gctgtagaactccaccacgc

SEQ ID NO: 106 - DNA, 20 bp, Artificial
  sgRNA
aatcatctgctacggacaac